European Patent Specification EP 4 182 337 B1, published December 17, 2025. Title: CHIMERIC MYD88 RECEPTORS FOR REDIRECTING IMMUNOSUPPRESSIVE SIGNALING AND RELATED COMPOSITIONS AND METHODS. Applicant: Simurx, Inc. Children's Hospital Los Angeles. Application Not Yet Assigned. The sequence listing filed with the application follows.

SEQUENCE LISTING (130 sequences)

SEQ ID NO: 1 - protein, 150 aa, Artificial Sequence
  TGFBR1, amino acids 34-183 (ectodomain, amino acids 34-126; transmembrane domain, amino acids 127-147); portion of cytoplasmic domain, amino acids 148-183)
LQCFCHLCTKDNFTCVTDGLCFVSVTETTDKVIHNSMCIAEIDLIPRDRPFVCAPSSKTGSVTTTYCCNQDHCNKIELPTTVKSSPGLGPVELAAVIAGPVCFVCISLMLMVYICHNRTVIHHRVPNEEDPSLDRPFISEGTTLKDLIYD

SEQ ID NO: 2 - protein, 170 aa, Artificial Sequence
  MYD88, amino acids 2-171
AAGGPGAGSAAPVSSTSSLPLAALNMRVRRRLSLFLNVRTQVAADWTALAEEMDFEYLEIRQLETQADPTGRLLDAWQGRPGASVGRLLELLTKLGRDDVLLELGPSIEEDCQKYILKQQQEEAEKPLQVAAVDSSVPRTAELAGITTLDDPLGHMPERFDAFICYCPSD

SEQ ID NO: 3 - protein, 176 aa, Artificial Sequence
  TGFBR2
TIPPHVQKSVNNDMIVTDNNGAVKFPQLCKFCDVRFSTCDNQKSCMSNCSITSICEKPQEVCVAVWRKNDENITLETVCHDPKLPYHDFILEDAASPKCIMKEKKKPGETFFMCSCSSDECNDNIIFSEEYNTSNPDLLLVIFQVTGISLLPPLGVAISVIIIFYCYRVNRQQKLS

SEQ ID NO: 4 - protein, 93 aa, Artificial Sequence
  TGFBR1 Extracellular
LQCFCHLCTKDNFTCVTDGLCFVSVTETTDKVIHNSMCIAEIDLIPRDRPFVCAPSSKTGSVTTTYCCNQDHCNKIELPTTVKSSPGLGPVEL

SEQ ID NO: 5 - DNA, 279 bp, Artificial Sequence
  TGFBR1 Extracellular
ctgcaatgtttttgtcacctctgtacgaaagataattttacgtgtgtcactgatggcctttgttttgtctcagtcactgaaactacggataaagtaatacataatagcatgtgtattgcagagattgatctcatcccgagagaccggcctttcgtctgtgcgcctagctccaaaacaggatcagttaccaccacgtattgctgtaaccaagaccactgcaacaaaatcgagcttccaacaactgtaaagtcttcccctggccttggccctgtagaactg

SEQ ID NO: 6 - protein, 21 aa, Artificial Sequence
  TGFBR1 Transmembrane
AAVIAGPVCFVCISLMLMVYI

SEQ ID NO: 7 - DNA, 63 bp, Artificial Sequence
  TGFBR1 Transmembrane
gctgcggtaattgctgggcccgtatgctttgtttgtatctccctcatgctcatggtctacatc

SEQ ID NO: 8 - protein, 36 aa, Artificial Sequence
  TGFBR1 Intracellular
CHNRTVIHHRVPNEEDPSLDRPFISEGTTLKDLIYD

SEQ ID NO: 9 - DNA, 108 bp, Artificial Sequence
  TGFBR1 Intracellular
tgtcataaccgcacggtcatacaccatcgcgtgcctaatgaagaggatccatcactcgatcggccttttatttctgagggcactactcttaaagacttgatctatgac

SEQ ID NO: 10 - protein, 108 aa, Artificial Sequence
  MYD88 DD
AAGGPGAGSAAPVSSTSSLPLAALNMRVRRRLSLFLNVRTQVAADWTALAEEMDFEYLEIRQLETQADPTGRLLDAWQGRPGASVGRLLELLTKLGRDDVLLELGPSI

SEQ ID NO: 11 - DNA, 324 bp, Artificial Sequence
  MYD88 DD
gcggctggcggaccaggggcaggttcagctgctccagtaagtagcacctcctcattgcctttggctgcattgaatatgcgggtacggagaagacttagtctcttcttgaacgtaagaactcaagtcgccgcagattggacggctcttgccgaagaaatggactttgaatatctcgagattcgacaactcgaaacccaagcggatccaactggtcggttgcttgacgcttggcagggtcgccctggagcgtctgtcggccgattgcttgaattgttgacaaaacttggcagagatgacgtgctcctggaactcggcccctccatc

SEQ ID NO: 12 - protein, 49 aa, Artificial Sequence
  MYD88 ID
EEDCQKYILKQQQEEAEKPLQVAAVDSSVPRTAELAGITTLDDPLGHMP

SEQ ID NO: 13 - DNA, 147 bp, Artificial Sequence
  MYD88 ID
gaagaggactgtcagaaatacattctgaaacagcaacaagaggaagcggaaaagcccctgcaggtcgctgcagttgattctagcgttcctcggaccgcggaacttgcaggcataaccactctcgacgatcccttggggcacatgcct

SEQ ID NO: 14 - protein, 13 aa, Artificial Sequence
  MYD88 TIR
ERFDAFICYCPSD

SEQ ID NO: 15 - DNA, 39 bp, Artificial Sequence
  MYD88 TIR
gaacgctttgacgccttcatttgttattgcccaagcgac

SEQ ID NO: 16 - protein, 347 aa, Artificial Sequence
  CTSR-1A
MALPVTALLLPLALLLHAARPHHHHHHLQCFCHLCTKDNFTCVTDGLCFVSVTETTDKVIHNSMCIAEIDLIPRDRPFVCAPSSKTGSVTTTYCCNQDHCNKIELPTTVKSSPGLGPVELAAVIAGPVCFVCISLMLMVYICHNRTVIHHRVPNEEDPSLDRPFISEGTTLKDLIYDAAGGPGAGSAAPVSSTSSLPLAALNMRVRRRLSLFLNVRTQVAADWTALAEEMDFEYLEIRQLETQADPTGRLLDAWQGRPGASVGRLLELLTKLGRDDVLLELGPSIEEDCQKYILKQQQEEAEKPLQVAAVDSSVPRTAELAGITTLDDPLGHMPERFDAFICYCPSD

SEQ ID NO: 17 - DNA, 1044 bp, Artificial Sequence
  CTSR-1A
atggcacttcccgttacagcactgctcctgcccctggcgctgctcctgcacgcggcccgcccccatcatcaccatcaccacctgcaatgtttttgtcacctctgtacgaaagataattttacgtgtgtcactgatggcctttgttttgtctcagtcactgaaactacggataaagtaatacataatagcatgtgtattgcagagattgatctcatcccgagagaccggcctttcgtctgtgcgcctagctccaaaacaggatcagttaccaccacgtattgctgtaaccaagaccactgcaacaaaatcgagcttccaacaactgtaaagtcttcccctggccttggccctgtagaactggctgcggtaattgctgggcccgtatgctttgtttgtatctccctcatgctcatggtctacatctgtcataaccgcacggtcatacaccatcgcgtgcctaatgaagaggatccatcactcgatcggccttttatttctgagggcactactcttaaagacttgatctatgacgcggctggcggaccaggggcaggttcagctgctccagtaagtagcacctcctcattgcctttggctgcattgaatatgcgggtacggagaagacttagtctcttcttgaacgtaagaactcaagtcgccgcagattggacggctcttgccgaagaaatggactttgaatatctcgagattcgacaactcgaaacccaagcggatccaactggtcggttgcttgacgcttggcagggtcgccctggagcgtctgtcggccgattgcttgaattgttgacaaaacttggcagagatgacgtgctcctggaactcggcccctccatcgaagaggactgtcagaaatacattctgaaacagcaacaagaggaagcggaaaagcccctgcaggtcgctgcagttgattctagcgttcctcggaccgcggaacttgcaggcataaccactctcgacgatcccttggggcacatgcctgaacgctttgacgccttcatttgttattgcccaagcgactag

SEQ ID NO: 18 - protein, 321 aa, Artificial Sequence
  CTSR-1B
MALPVTALLLPLALLLHAARPHHHHHHLQCFCHLCTKDNFTCVTDGLCFVSVTETTDKVIHNSMCIAEIDLIPRDRPFVCAPSSKTGSVTTTYCCNQDHCNKIELPTTVKSSPGLGPVELAAVIAGPVCFVCISLMLMVYIGGGGSGGGGSAAGGPGAGSAAPVSSTSSLPLAALNMRVRRRLSLFLNVRTQVAADWTALAEEMDFEYLEIRQLETQADPTGRLLDAWQGRPGASVGRLLELLTKLGRDDVLLELGPSIEEDCQKYILKQQQEEAEKPLQVAAVDSSVPRTAELAGITTLDDPLGHMPERFDAFICYCPSD

SEQ ID NO: 19 - DNA, 966 bp, Artificial Sequence
  CTSR-1B
atggcacttcccgttacagcactgctcctgcccctggcgctgctcctgcacgcggcccgcccccatcatcaccatcaccacctgcaatgtttttgtcacctctgtacgaaagataattttacgtgtgtcactgatggcctttgttttgtctcagtcactgaaactacggataaagtaatacataatagcatgtgtattgcagagattgatctcatcccgagagaccggcctttcgtctgtgcgcctagctccaaaacaggatcagttaccaccacgtattgctgtaaccaagaccactgcaacaaaatcgagcttccaacaactgtaaagtcttcccctggccttggccctgtagaactggctgcggtaattgctgggcccgtatgctttgtttgtatctccctcatgctcatggtctacatcggcggcggtggtagcggtggcggtggcagcgcggctggcggaccaggggcaggttcagctgctccagtaagtagcacctcctcattgcctttggctgcattgaatatgcgggtacggagaagacttagtctcttcttgaacgtaagaactcaagtcgccgcagattggacggctcttgccgaagaaatggactttgaatatctcgagattcgacaactcgaaacccaagcggatccaactggtcggttgcttgacgcttggcagggtcgccctggagcgtctgtcggccgattgcttgaattgttgacaaaacttggcagagatgacgtgctcctggaactcggcccctccatcgaagaggactgtcagaaatacattctgaaacagcaacaagaggaagcggaaaagcccctgcaggtcgctgcagttgattctagcgttcctcggaccgcggaacttgcaggcataaccactctcgacgatcccttggggcacatgcctgaacgctttgacgccttcatttgttattgcccaagcgactag

SEQ ID NO: 20 - protein, 144 aa, Artificial Sequence
  TGFBR2 Extracellular domain
TIPPHVQKSVNNDMIVTDNNGAVKFPQLCKFCDVRFSTCDNQKSCMSNCSITSICEKPQEVCVAVWRKNDENITLETVCHDPKLPYHDFILEDAASPKCIMKEKKKPGETFFMCSCSSDECNDNIIFSEEYNTSNPDLLLVIFQ

SEQ ID NO: 21 - DNA, 432 bp, Artificial Sequence
  TGFBR2 Extracellular domain
actattccccctcatgttcagaaatccgtaaacaatgatatgattgtcacggacaacaacggtgcggtcaaattcccgcagctttgcaaattttgtgatgttagattctcaacgtgtgataatcaaaagtcctgcatgagtaattgttcaattacttccatctgcgaaaagcctcaggaagtttgcgtcgcagtctggaggaagaacgacgaaaacattacacttgagactgtgtgtcatgatcctaaactcccctatcatgacttcatccttgaggatgcggcgtcccccaaatgtatcatgaaagagaaaaaaaagcccggtgagacgttcttcatgtgcagctgctccagcgacgagtgcaatgataacatcattttctctgaagaatacaatacctcaaatcccgacctcctcttggtaatatttcag

SEQ ID NO: 22 - protein, 21 aa, Artificial Sequence
  TGFBR2 Transmembrane
VTGISLLPPLGVAISVIIIFY

SEQ ID NO: 23 - DNA, 63 bp, Artificial Sequence
  TGFBR2 Transmembrane
gtgacgggtataagtttgcttccgcctctcggtgtggcgatctccgttatcattatcttttat

SEQ ID NO: 24 - protein, 11 aa, Artificial Sequence
  TGFBR2 Cytoplasmic domain
CYRVNRQQKLS

SEQ ID NO: 25 - DNA, 33 bp, Artificial Sequence
  TGFBR2 Cytoplasmic domain
tgctatcgcgtgaacagacaacaaaaattgtcc

SEQ ID NO: 26 - protein, 377 aa, Artificial Sequence
  CTSR-2A
MALPVTALLLPLALLLHAARPEQKLISEEDLTIPPHVQKSVNNDMIVTDNNGAVKFPQLCKFCDVRFSTCDNQKSCMSNCSITSICEKPQEVCVAVWRKNDENITLETVCHDPKLPYHDFILEDAASPKCIMKEKKKPGETFFMCSCSSDECNDNIIFSEEYNTSNPDLLLVIFQVTGISLLPPLGVAISVIIIFYCYRVNRQQKLSAAGGPGAGSAAPVSSTSSLPLAALNMRVRRRLSLFLNVRTQVAADWTALAEEMDFEYLEIRQLETQADPTGRLLDAWQGRPGASVGRLLELLTKLGRDDVLLELGPSIEEDCQKYILKQQQEEAEKPLQVAAVDSSVPRTAELAGITTLDDPLGHMPERFDAFICYCPSD

SEQ ID NO: 27 - DNA, 1134 bp, Artificial Sequence
  CTSR-2A
atggcacttcccgttacagcactgctcctgcccctggcgctgctcctgcacgcggcccgccccgagcaaaaacttatctctgaagaggacctcactattccccctcatgttcagaaatccgtaaacaatgatatgattgtcacggacaacaacggtgcggtcaaattcccgcagctttgcaaattttgtgatgttagattctcaacgtgtgataatcaaaagtcctgcatgagtaattgttcaattacttccatctgcgaaaagcctcaggaagtttgcgtcgcagtctggaggaagaacgacgaaaacattacacttgagactgtgtgtcatgatcctaaactcccctatcatgacttcatccttgaggatgcggcgtcccccaaatgtatcatgaaagagaaaaaaaagcccggtgagacgttcttcatgtgcagctgctccagcgacgagtgcaatgataacatcattttctctgaagaatacaatacctcaaatcccgacctcctcttggtaatatttcaggtgacgggtataagtttgcttccgcctctcggtgtggcgatctccgttatcattatcttttattgctatcgcgtgaacagacaacaaaaattgtccgcggctggcggaccaggggcaggttcagctgctccagtaagtagcacctcctcattgcctttggctgcattgaatatgcgggtacggagaagacttagtctcttcttgaacgtaagaactcaagtcgccgcagattggacggctcttgccgaagaaatggactttgaatatctcgagattcgacaactcgaaacccaagcggatccaactggtcggttgcttgacgcttggcagggtcgccctggagcgtctgtcggccgattgcttgaattgttgacaaaacttggcagagatgacgtgctcctggaactcggcccctccatcgaagaggactgtcagaaatacattctgaaacagcaacaagaggaagcggaaaagcccctgcaggtcgctgcagttgattctagcgttcctcggaccgcggaacttgcaggcataaccactctcgacgatcccttggggcacatgcctgaacgctttgacgccttcatttgttattgcccaagcgactag

SEQ ID NO: 28 - protein, 547 aa, Artificial Sequence
  CTSR-2B
MALPVTALLLPLALLLHAARPEQKLISEEDLTIPPHVQKSVNNDMIVTDNNGAVKFPQLCKFCDVRFSTCDNQKSCMSNCSITSICEKPQEVCVAVWRKNDENITLETVCHDPKLPYHDFILEDAASPKCIMKEKKKPGETFFMCSCSSDECNDNIIFSEEYNTSNPDLLLVIFQVTGISLLPPLGVAISVIIIFYCYRVNRQQKLSAAGGPGAGSAAPVSSTSSLPLAALNMRVRRRLSLFLNVRTQVAADWTALAEEMDFEYLEIRQLETQADPTGRLLDAWQGRPGASVGRLLELLTKLGRDDVLLELGPSIEEDCQKYILKQQQEEAEKPLQVAAVDSSVPRTAELAGITTLDDPLGHMPERFDAFICYCPSDAAGGPGAGSAAPVSSTSSLPLAALNMRVRRRLSLFLNVRTQVAADWTALAEEMDFEYLEIRQLETQADPTGRLLDAWQGRPGASVGRLLELLTKLGRDDVLLELGPSIEEDCQKYILKQQQEEAEKPLQVAAVDSSVPRTAELAGITTLDDPLGHMPERFDAFICYCPSD

SEQ ID NO: 29 - DNA, 1644 bp, Artificial Sequence
  CTSR-2B
atggcacttcccgttacagcactgctcctgcccctggcgctgctcctgcacgcggcccgccccgagcaaaaacttatctctgaagaggacctcactattccccctcatgttcagaaatccgtaaacaatgatatgattgtcacggacaacaacggtgcggtcaaattcccgcagctttgcaaattttgtgatgttagattctcaacgtgtgataatcaaaagtcctgcatgagtaattgttcaattacttccatctgcgaaaagcctcaggaagtttgcgtcgcagtctggaggaagaacgacgaaaacattacacttgagactgtgtgtcatgatcctaaactcccctatcatgacttcatccttgaggatgcggcgtcccccaaatgtatcatgaaagagaaaaaaaagcccggtgagacgttcttcatgtgcagctgctccagcgacgagtgcaatgataacatcattttctctgaagaatacaatacctcaaatcccgacctcctcttggtaatatttcaggtgacgggtataagtttgcttccgcctctcggtgtggcgatctccgttatcattatcttttattgctatcgcgtgaacagacaacaaaaattgtccgcggctggcggaccaggggcaggttcagctgctccagtaagtagcacctcctcattgcctttggctgcattgaatatgcgggtacggagaagacttagtctcttcttgaacgtaagaactcaagtcgccgcagattggacggctcttgccgaagaaatggactttgaatatctcgagattcgacaactcgaaacccaagcggatccaactggtcggttgcttgacgcttggcagggtcgccctggagcgtctgtcggccgattgcttgaattgttgacaaaacttggcagagatgacgtgctcctggaactcggcccctccatcgaagaggactgtcagaaatacattctgaaacagcaacaagaggaagcggaaaagcccctgcaggtcgctgcagttgattctagcgttcctcggaccgcggaacttgcaggcataaccactctcgacgatcccttggggcacatgcctgaacgctttgacgccttcatttgttattgcccaagcgacgcggctggcggaccaggggcaggttcagctgctccagtaagtagcacctcctcattgcctttggctgcattgaatatgcgggtacggagaagacttagtctcttcttgaacgtaagaactcaagtcgccgcagattggacggctcttgccgaagaaatggactttgaatatctcgagattcgacaactcgaaacccaagcggatccaactggtcggttgcttgacgcttggcagggtcgccctggagcgtctgtcggccgattgcttgaattgttgacaaaacttggcagagatgacgtgctcctggaactcggcccctccatcgaagaggactgtcagaaatacattctgaaacagcaacaagaggaagcggaaaagcccctgcaggtcgctgcagttgattctagcgttcctcggaccgcggaacttgcaggcataaccactctcgacgatcccttggggcacatgcctgaacgctttgacgccttcatttgttattgcccaagcgactag

SEQ ID NO: 30 - protein, 552 aa, Artificial Sequence
  CTSR-2C
MALPVTALLLPLALLLHAARPEQKLISEEDLTIPPHVQKSVNNDMIVTDNNGAVKFPQLCKFCDVRFSTCDNQKSCMSNCSITSICEKPQEVCVAVWRKNDENITLETVCHDPKLPYHDFILEDAASPKCIMKEKKKPGETFFMCSCSSDECNDNIIFSEEYNTSNPDLLLVIFQVTGISLLPPLGVAISVIIIFYCYRVNRQQKLSAAGGPGAGSAAPVSSTSSLPLAALNMRVRRRLSLFLNVRTQVAADWTALAEEMDFEYLEIRQLETQADPTGRLLDAWQGRPGASVGRLLELLTKLGRDDVLLELGPSIEEDCQKYILKQQQEEAEKPLQVAAVDSSVPRTAELAGITTLDDPLGHMPERFDAFICYCPSDGGGGSAAGGPGAGSAAPVSSTSSLPLAALNMRVRRRLSLFLNVRTQVAADWTALAEEMDFEYLEIRQLETQADPTGRLLDAWQGRPGASVGRLLELLTKLGRDDVLLELGPSIEEDCQKYILKQQQEEAEKPLQVAAVDSSVPRTAELAGITTLDDPLGHMPERFDAFICYCPSD

SEQ ID NO: 31 - DNA, 1659 bp, Artificial Sequence
  CTSR-2C
atggcacttcccgttacagcactgctcctgcccctggcgctgctcctgcacgcggcccgccccgagcaaaaacttatctctgaagaggacctcactattccccctcatgttcagaaatccgtaaacaatgatatgattgtcacggacaacaacggtgcggtcaaattcccgcagctttgcaaattttgtgatgttagattctcaacgtgtgataatcaaaagtcctgcatgagtaattgttcaattacttccatctgcgaaaagcctcaggaagtttgcgtcgcagtctggaggaagaacgacgaaaacattacacttgagactgtgtgtcatgatcctaaactcccctatcatgacttcatccttgaggatgcggcgtcccccaaatgtatcatgaaagagaaaaaaaagcccggtgagacgttcttcatgtgcagctgctccagcgacgagtgcaatgataacatcattttctctgaagaatacaatacctcaaatcccgacctcctcttggtaatatttcaggtgacgggtataagtttgcttccgcctctcggtgtggcgatctccgttatcattatcttttattgctatcgcgtgaacagacaacaaaaattgtccgcggctggcggaccaggggcaggttcagctgctccagtaagtagcacctcctcattgcctttggctgcattgaatatgcgggtacggagaagacttagtctcttcttgaacgtaagaactcaagtcgccgcagattggacggctcttgccgaagaaatggactttgaatatctcgagattcgacaactcgaaacccaagcggatccaactggtcggttgcttgacgcttggcagggtcgccctggagcgtctgtcggccgattgcttgaattgttgacaaaacttggcagagatgacgtgctcctggaactcggcccctccatcgaagaggactgtcagaaatacattctgaaacagcaacaagaggaagcggaaaagcccctgcaggtcgctgcagttgattctagcgttcctcggaccgcggaacttgcaggcataaccactctcgacgatcccttggggcacatgcctgaacgctttgacgccttcatttgttattgcccaagcgacggtggcggtggctcggcggctggcggaccaggggcaggttcagctgctccagtaagtagcacctcctcattgcctttggctgcattgaatatgcgggtacggagaagacttagtctcttcttgaacgtaagaactcaagtcgccgcagattggacggctcttgccgaagaaatggactttgaatatctcgagattcgacaactcgaaacccaagcggatccaactggtcggttgcttgacgcttggcagggtcgccctggagcgtctgtcggccgattgcttgaattgttgacaaaacttggcagagatgacgtgctcctggaactcggcccctccatcgaagaggactgtcagaaatacattctgaaacagcaacaagaggaagcggaaaagcccctgcaggtcgctgcagttgattctagcgttcctcggaccgcggaacttgcaggcataaccactctcgacgatcccttggggcacatgcctgaacgctttgacgccttcatttgttattgcccaagcgactag

SEQ ID NO: 32 - protein, 200 aa, Artificial Sequence
  CTSR-2IN
MALPVTALLLPLALLLHAARPEQKLISEEDLTIPPHVQKSVNNDMIVTDNNGAVKFPQLCKFCDVRFSTCDNQKSCMSNCSITSICEKPQEVCVAVWRKNDENITLETVCHDPKLPYHDFILEDAASPKCIMKEKKKPGETFFMCSCSSDECNDNIIFSEEYNTSNPDLLLVIFQVTGISLLPPLGVAISVIIIFYCYRV

SEQ ID NO: 33 - DNA, 603 bp, Artificial Sequence
  CTSR-2IN
atggcacttcccgttacagcactgctcctgcccctggcgctgctcctgcacgcggcccgccccgagcaaaaacttatctctgaagaggacctcactattccccctcatgttcagaaatccgtaaacaatgatatgattgtcacggacaacaacggtgcggtcaaattcccgcagctttgcaaattttgtgatgttagattctcaacgtgtgataatcaaaagtcctgcatgagtaattgttcaattacttccatctgcgaaaagcctcaggaagtttgcgtcgcagtctggaggaagaacgacgaaaacattacacttgagactgtgtgtcatgatcctaaactcccctatcatgacttcatccttgaggatgcggcgtcccccaaatgtatcatgaaagagaaaaaaaagcccggtgagacgttcttcatgtgcagctgctccagcgacgagtgcaatgataacatcattttctctgaagaatacaatacctcaaatcccgacctcctcttggtaatatttcaggtgacgggtataagtttgcttccgcctctcggtgtggcgatctccgttatcattatcttttattgctatcgcgtgtag

SEQ ID NO: 34 - protein, 230 aa, Artificial Sequence
  CTSR-2IN-T2A
MALPVTALLLPLALLLHAARPEQKLISEEDLTIPPHVQKSVNNDMIVTDNNGAVKFPQLCKFCDVRFSTCDNQKSCMSNCSITSICEKPQEVCVAVWRKNDENITLETVCHDPKLPYHDFILEDAASPKCIMKEKKKPGETFFMCSCSSDECNDNIIFSEEYNTSNPDLLLVIFQVTGISLLPPLGVAISVIIIFYCYRVNRQQKLSAAGSGEGRGSLLTCGDVEENPGP

SEQ ID NO: 35 - DNA, 690 bp, Artificial Sequence
  CTSR-2IN-T2A
atggcacttcccgttacagcactgctcctgcccctggcgctgctcctgcacgcggcccgccccgagcaaaaacttatctctgaagaggacctcactattccccctcatgttcagaaatccgtaaacaatgatatgattgtcacggacaacaacggtgcggtcaaattcccgcagctttgcaaattttgtgatgttagattctcaacgtgtgataatcaaaagtcctgcatgagtaattgttcaattacttccatctgcgaaaagcctcaggaagtttgcgtcgcagtctggaggaagaacgacgaaaacattacacttgagactgtgtgtcatgatcctaaactcccctatcatgacttcatccttgaggatgcggcgtcccccaaatgtatcatgaaagagaaaaaaaagcccggtgagacgttcttcatgtgcagctgctccagcgacgagtgcaatgataacatcattttctctgaagaatacaatacctcaaatcccgacctcctcttggtaatatttcaggtgacgggtataagtttgcttccgcctctcggtgtggcgatctccgttatcattatcttttattgctatcgcgtgaacagacaacaaaaattgtccgcggctggatctggtgaggggcgggggtccctgctgacctgcggcgacgtcgaagaaaatcccggtccc

SEQ ID NO: 36 - protein, 421 aa, Artificial Sequence
  CTSR-2EN
MALPVTALLLPLALLLHAARPEQKLISEEDLTIPPHVQKSVNNDVTGISLLPPLGVAISVIIIFYCYRVNRQQKLSAAGGPGAGSAAPVSSTSSLPLAALNMRVRRRLSLFLNVRTQVAADWTALAEEMDFEYLEIRQLETQADPTGRLLDAWQGRPGASVGRLLELLTKLGRDDVLLELGPSIEEDCQKYILKQQQEEAEKPLQVAAVDSSVPRTAELAGITTLDDPLGHMPERFDAFICYCPSDGGGGSAAGGPGAGSAAPVSSTSSLPLAALNMRVRRRLSLFLNVRTQVAADWTALAEEMDFEYLEIRQLETQADPTGRLLDAWQGRPGASVGRLLELLTKLGRDDVLLELGPSIEEDCQKYILKQQQEEAEKPLQVAAVDSSVPRTAELAGITTLDDPLGHMPERFDAFICYCPSD

SEQ ID NO: 37 - DNA, 1263 bp, Artificial Sequence
  CTSR-2EN
atggcacttcccgttacagcactgctcctgcccctggcgctgctcctgcacgcggcccgccccgagcaaaaacttatctctgaagaggacctcactattccccctcatgttcagaaatccgtaaacaatgatgtgacgggtataagtttgcttccgcctctcggtgtggcgatctccgttatcattatcttttattgctatcgcgtgaacagacaacaaaaattgtccgcggctggcggaccaggggcaggttcagctgctccagtaagtagcacctcctcattgcctttggctgcattgaatatgcgggtacggagaagacttagtctcttcttgaacgtaagaactcaagtcgccgcagattggacggctcttgccgaagaaatggactttgaatatctcgagattcgacaactcgaaacccaagcggatccaactggtcggttgcttgacgcttggcagggtcgccctggagcgtctgtcggccgattgcttgaattgttgacaaaacttggcagagatgacgtgctcctggaactcggcccctccatcgaagaggactgtcagaaatacattctgaaacagcaacaagaggaagcggaaaagcccctgcaggtcgctgcagttgattctagcgttcctcggaccgcggaacttgcaggcataaccactctcgacgatcccttggggcacatgcctgaacgctttgacgccttcatttgttattgcccaagcgacggtggcggtggctcggcggctggcggaccaggggcaggttcagctgctccagtaagtagcacctcctcattgcctttggctgcattgaatatgcgggtacggagaagacttagtctcttcttgaacgtaagaactcaagtcgccgcagattggacggctcttgccgaagaaatggactttgaatatctcgagattcgacaactcgaaacccaagcggatccaactggtcggttgcttgacgcttggcagggtcgccctggagcgtctgtcggccgattgcttgaattgttgacaaaacttggcagagatgacgtgctcctggaactcggcccctccatcgaagaggactgtcagaaatacattctgaaacagcaacaagaggaagcggaaaagcccctgcaggtcgctgcagttgattctagcgttcctcggaccgcggaacttgcaggcataaccactctcgacgatcccttggggcacatgcctgaacgctttgacgccttcatttgttattgcccaagcgac

SEQ ID NO: 38 - protein, 486 aa, Artificial Sequence
  CAR-B
MALPVTALLLPLALLLHAARPDIQMTQTTSSLSASLGDRVTISCRASQDISKYLNWYQQKPDGTVKLLIYHTSRLHSGVPSRFSGSGSGTDYSLTISNLEQEDIATYFCQQGNTLPYTFGGGTKLEITGGGGSGGGGSGGGGSEVKLQESGPGLVAPSQSLSVTCTVSGVSLPDYGVSWIRQPPRKGLEWLGVIWGSETTYYNSALKSRLTIIKDNSKSQVFLKMNSLQTDDTAIYYCAKHYYYGGSYAMDYWGQGTSVTVSSTTTPAPRPPTPAPTIASQPLSLRPEACRPAAGGAVHTRGLDFACDIYIWAPLAGTCGVLLLSLVITLYCKRGRKKLLYIFKQPFMRPVQTTQEEDGCSCRFPEEEEGGCELRVKFSRSADAPAYKQGQNQLYNELNLGRREEYDVLDKRRGRDPEMGGKPRRKNPQEGLYNELQKDKMAEAYSEIGMKGERRRGKGHDGLYQGLSTATKDTYDALHMQALPPR

SEQ ID NO: 39 - protein, 573 aa, Artificial Sequence
  CTSR-2C-T2A
MALPVTALLLPLALLLHAARPEQKLISEEDLTIPPHVQKSVNNDMIVTDNNGAVKFPQLCKFCDVRFSTCDNQKSCMSNCSITSICEKPQEVCVAVWRKNDENITLETVCHDPKLPYHDFILEDAASPKCIMKEKKKPGETFFMCSCSSDECNDNIIFSEEYNTSNPDLLLVIFQVTGISLLPPLGVAISVIIIFYCYRVNRQQKLSAAGGPGAGSAAPVSSTSSLPLAALNMRVRRRLSLFLNVRTQVAADWTALAEEMDFEYLEIRQLETQADPTGRLLDAWQGRPGASVGRLLELLTKLGRDDVLLELGPSIEEDCQKYILKQQQEEAEKPLQVAAVDSSVPRTAELAGITTLDDPLGHMPERFDAFICYCPSDGGGGSAAGGPGAGSAAPVSSTSSLPLAALNMRVRRRLSLFLNVRTQVAADWTALAEEMDFEYLEIRQLETQADPTGRLLDAWQGRPGASVGRLLELLTKLGRDDVLLELGPSIEEDCQKYILKQQQEEAEKPLQVAAVDSSVPRTAELAGITTLDDPLGHMPERFDAFICYCPSDGSGEGRGSLLTCGDVEENPGP

SEQ ID NO: 40 - DNA, 1719 bp, Artificial Sequence
  CTSR-2C-T2A
atggcacttcccgttacagcactgctcctgcccctggcgctgctcctgcacgcggcccgccccgagcaaaaacttatctctgaagaggacctcactattccccctcatgttcagaaatccgtaaacaatgatatgattgtcacggacaacaacggtgcggtcaaattcccgcagctttgcaaattttgtgatgttagattctcaacgtgtgataatcaaaagtcctgcatgagtaattgttcaattacttccatctgcgaaaagcctcaggaagtttgcgtcgcagtctggaggaagaacgacgaaaacattacacttgagactgtgtgtcatgatcctaaactcccctatcatgacttcatccttgaggatgcggcgtcccccaaatgtatcatgaaagagaaaaaaaagcccggtgagacgttcttcatgtgcagctgctccagcgacgagtgcaatgataacatcattttctctgaagaatacaatacctcaaatcccgacctcctcttggtaatatttcaggtgacgggtataagtttgcttccgcctctcggtgtggcgatctccgttatcattatcttttattgctatcgcgtgaacagacaacaaaaattgtccgcggctggcggaccaggggcaggttcagctgctccagtaagtagcacctcctcattgcctttggctgcattgaatatgcgggtacggagaagacttagtctcttcttgaacgtaagaactcaagtcgccgcagattggacggctcttgccgaagaaatggactttgaatatctcgagattcgacaactcgaaacccaagcggatccaactggtcggttgcttgacgcttggcagggtcgccctggagcgtctgtcggccgattgcttgaattgttgacaaaacttggcagagatgacgtgctcctggaactcggcccctccatcgaagaggactgtcagaaatacattctgaaacagcaacaagaggaagcggaaaagcccctgcaggtcgctgcagttgattctagcgttcctcggaccgcggaacttgcaggcataaccactctcgacgatcccttggggcacatgcctgaacgctttgacgccttcatttgttattgcccaagcgacggtggcggtggctcggcggctggcggaccaggggcaggttcagctgctccagtaagtagcacctcctcattgcctttggctgcattgaatatgcgggtacggagaagacttagtctcttcttgaacgtaagaactcaagtcgccgcagattggacggctcttgccgaagaaatggactttgaatatctcgagattcgacaactcgaaacccaagcggatccaactggtcggttgcttgacgcttggcagggtcgccctggagcgtctgtcggccgattgcttgaattgttgacaaaacttggcagagatgacgtgctcctggaactcggcccctccatcgaagaggactgtcagaaatacattctgaaacagcaacaagaggaagcggaaaagcccctgcaggtcgctgcagttgattctagcgttcctcggaccgcggaacttgcaggcataaccactctcgacgatcccttggggcacatgcctgaacgctttgacgccttcatttgttattgcccaagcgacggatctggtgaggggcgggggtccctgctgacctgcggcgacgtcgaagaaaatcccggtccc

SEQ ID NO: 41 - protein, 398 aa, Artificial Sequence
  CTSR-2A-T2A
MALPVTALLLPLALLLHAARPEQKLISEEDLTIPPHVQKSVNNDMIVTDNNGAVKFPQLCKFCDVRFSTCDNQKSCMSNCSITSICEKPQEVCVAVWRKNDENITLETVCHDPKLPYHDFILEDAASPKCIMKEKKKPGETFFMCSCSSDECNDNIIFSEEYNTSNPDLLLVIFQVTGISLLPPLGVAISVIIIFYCYRVNRQQKLSAAGGPGAGSAAPVSSTSSLPLAALNMRVRRRLSLFLNVRTQVAADWTALAEEMDFEYLEIRQLETQADPTGRLLDAWQGRPGASVGRLLELLTKLGRDDVLLELGPSIEEDCQKYILKQQQEEAEKPLQVAAVDSSVPRTAELAGITTLDDPLGHMPERFDAFICYCPSDGSGEGRGSLLTCGDVEENPGP

SEQ ID NO: 42 - DNA, 1194 bp, Artificial Sequence
  CTSR-2A-T2A
atggcacttcccgttacagcactgctcctgcccctggcgctgctcctgcacgcggcccgccccgagcaaaaacttatctctgaagaggacctcactattccccctcatgttcagaaatccgtaaacaatgatatgattgtcacggacaacaacggtgcggtcaaattcccgcagctttgcaaattttgtgatgttagattctcaacgtgtgataatcaaaagtcctgcatgagtaattgttcaattacttccatctgcgaaaagcctcaggaagtttgcgtcgcagtctggaggaagaacgacgaaaacattacacttgagactgtgtgtcatgatcctaaactcccctatcatgacttcatccttgaggatgcggcgtcccccaaatgtatcatgaaagagaaaaaaaagcccggtgagacgttcttcatgtgcagctgctccagcgacgagtgcaatgataacatcattttctctgaagaatacaatacctcaaatcccgacctcctcttggtaatatttcaggtgacgggtataagtttgcttccgcctctcggtgtggcgatctccgttatcattatcttttattgctatcgcgtgaacagacaacaaaaattgtccgcggctggcggaccaggggcaggttcagctgctccagtaagtagcacctcctcattgcctttggctgcattgaatatgcgggtacggagaagacttagtctcttcttgaacgtaagaactcaagtcgccgcagattggacggctcttgccgaagaaatggactttgaatatctcgagattcgacaactcgaaacccaagcggatccaactggtcggttgcttgacgcttggcagggtcgccctggagcgtctgtcggccgattgcttgaattgttgacaaaacttggcagagatgacgtgctcctggaactcggcccctccatcgaagaggactgtcagaaatacattctgaaacagcaacaagaggaagcggaaaagcccctgcaggtcgctgcagttgattctagcgttcctcggaccgcggaacttgcaggcataaccactctcgacgatcccttggggcacatgcctgaacgctttgacgccttcatttgttattgcccaagcgacggatctggtgaggggcgggggtccctgctgacctgcggcgacgtcgaagaaaatcccggtccc

SEQ ID NO: 43 - protein, 442 aa, Artificial Sequence
  CTSR-2EN-T2A
MALPVTALLLPLALLLHAARPEQKLISEEDLTIPPHVQKSVNNDVTGISLLPPLGVAISVIIIFYCYRVNRQQKLSAAGGPGAGSAAPVSSTSSLPLAALNMRVRRRLSLFLNVRTQVAADWTALAEEMDFEYLEIRQLETQADPTGRLLDAWQGRPGASVGRLLELLTKLGRDDVLLELGPSIEEDCQKYILKQQQEEAEKPLQVAAVDSSVPRTAELAGITTLDDPLGHMPERFDAFICYCPSDGGGGSAAGGPGAGSAAPVSSTSSLPLAALNMRVRRRLSLFLNVRTQVAADWTALAEEMDFEYLEIRQLETQADPTGRLLDAWQGRPGASVGRLLELLTKLGRDDVLLELGPSIEEDCQKYILKQQQEEAEKPLQVAAVDSSVPRTAELAGITTLDDPLGHMPERFDAFICYCPSDGSGEGRGSLLTCGDVEENPGP

SEQ ID NO: 44 - DNA, 1326 bp, Artificial Sequence
  CTSR-2EN-T2A
atggcacttcccgttacagcactgctcctgcccctggcgctgctcctgcacgcggcccgccccgagcaaaaacttatctctgaagaggacctcactattccccctcatgttcagaaatccgtaaacaatgatgtgacgggtataagtttgcttccgcctctcggtgtggcgatctccgttatcattatcttttattgctatcgcgtgaacagacaacaaaaattgtccgcggctggcggaccaggggcaggttcagctgctccagtaagtagcacctcctcattgcctttggctgcattgaatatgcgggtacggagaagacttagtctcttcttgaacgtaagaactcaagtcgccgcagattggacggctcttgccgaagaaatggactttgaatatctcgagattcgacaactcgaaacccaagcggatccaactggtcggttgcttgacgcttggcagggtcgccctggagcgtctgtcggccgattgcttgaattgttgacaaaacttggcagagatgacgtgctcctggaactcggcccctccatcgaagaggactgtcagaaatacattctgaaacagcaacaagaggaagcggaaaagcccctgcaggtcgctgcagttgattctagcgttcctcggaccgcggaacttgcaggcataaccactctcgacgatcccttggggcacatgcctgaacgctttgacgccttcatttgttattgcccaagcgacggtggcggtggctcggcggctggcggaccaggggcaggttcagctgctccagtaagtagcacctcctcattgcctttggctgcattgaatatgcgggtacggagaagacttagtctcttcttgaacgtaagaactcaagtcgccgcagattggacggctcttgccgaagaaatggactttgaatatctcgagattcgacaactcgaaacccaagcggatccaactggtcggttgcttgacgcttggcagggtcgccctggagcgtctgtcggccgattgcttgaattgttgacaaaacttggcagagatgacgtgctcctggaactcggcccctccatcgaagaggactgtcagaaatacattctgaaacagcaacaagaggaagcggaaaagcccctgcaggtcgctgcagttgattctagcgttcctcggaccgcggaacttgcaggcataaccactctcgacgatcccttggggcacatgcctgaacgctttgacgccttcatttgttattgcccaagcgacggatctggtgaggggcgggggtccctgctgacctgcggcgacgtcgaagaaaatcccggtccc

SEQ ID NO: 45 - protein, 493 aa, Artificial Sequence
  CAR-A
MALPVTALLLPLALLLHAARPDIAMTQSQKFMSTSVGDRVSVTCKASQNVDTNVAWYQQKPGQSPKALIYSASYRYSGVPDRFTGSGSGTDFTLTINNVQSEDLAEYFCQQYNNYPFTFGSGTKLEIKGGGGSGGGGSGGGGSGGGGSDVQLVESGGGLVQPGGSRKLSCAASGFTFSSFGMHWVRQAPEKGLEWVAYISSDSSAIYYADTVKGRFTISRDNPKNTLFLQMTSLRSEDTAMYYCGRGRENIYYGSRLDYWGQGTTLTVSSTTTPAPRPPTPAPTIASQPLSLRPEACRPAAGGAVHTRGLDFACDIYIWAPLAGTCGVLLLSLVITLYCKRGRKKLLYIFKQPFMRPVQTTQEEDGCSCRFPEEEEGGCELRVKFSRSADAPAYKQGQNQLYNELNLGRREEYDVLDKRRGRDPEMGGKPRRKNPQEGLYNELQKDKMAEAYSEIGMKGERRRGKGHDGLYQGLSTATKDTYDALHMQALPPR

SEQ ID NO: 46 - DNA, 1482 bp, Artificial Sequence
  CAR-A
atggccttaccagtgaccgccttgctcctgccgctggccttgctgctccacgccgccaggccggacatcgccatgacacaatctcaaaagttcatgtccacgtcagtcggagaccgagtctccgtcacttgcaaggccagtcagaatgtggataccaatgtagcatggtaccagcaaaaacccggacagtcacctaaggctcttatatactccgcttcttataggtattctggtgtacctgacaggtttactgggtccgggtccggcacagacttcactctgacaataaacaatgtgcaatcagaggacctcgcggagtatttctgtcagcaatataacaactacccatttactttcggttcaggcactaaactggagataaagggcggaggagggtcaggcgggggcggttcagggggaggtgggtcaggcggggggggttccgatgttcagttggtagagtccggggggggtctggtacagcctggtggatcaagaaaactgtcttgcgcggcgagtgggttcaccttctctagttttggaatgcactgggtacgccaagcaccggagaaaggtttggaatgggtcgcatacatttcttcagatagttcagcaatttattacgcggacacagtgaaaggacggtttacgatctccagagacaaccctaagaatacgctctttctccaaatgaccagcctccgatctgaagatacggcaatgtattattgtggtcggggcagagagaacatttattatggctcccgcctcgattactggggccaaggtaccactctgacggtctcttcaaccacgacgccagcgccgcgaccaccaacaccggcgcccaccatcgcgtcgcagcccctgtccctgcgcccagaggcgtgccggccagcggcggggggcgcagtgcacacgagggggctggacttcgcctgtgatatctacatctgggcgcccttggccgggacttgtggggtccttctcctgtcactggttatcaccctttactgcaaacggggcagaaagaaactcctgtatatattcaaacaaccatttatgagaccagtacaaactactcaagaggaagatggctgtagctgccgatttccagaagaagaagaaggaggatgtgaactgagagtgaagttcagcaggagcgcagacgcccccgcgtacaagcagggccagaaccagctctataacgagctcaatctaggacgaagagaggagtacgatgttttggacaagagacgtggccgggaccctgagatggggggaaagccgagaaggaagaaccctcaggaaggcctgtacaatgaactgcagaaagataagatggcggaggcctacagtgagattgggatgaaaggcgagcgccggaggggcaaggggcacgatggcctttaccagggtctcagtacagccaccaaggacacctacgacgcccttcacatgcaggccctgccccctcgctaa

SEQ ID NO: 47 - protein, 5 aa, Artificial Sequence
  Linker
  REPEAT (1)...(5): Repeats 1-4 times
GGGGS

SEQ ID NO: 48 - protein, 5 aa, Artificial Sequence
  Linker
GGGGS

SEQ ID NO: 49 - protein, 15 aa, Artificial Sequence
  Linker
GGGGSGGGGSGGGGS

SEQ ID NO: 50 - protein, 20 aa, Artificial Sequence
  Linker
GGGGSGGGGSGGGGSGGGGS

SEQ ID NO: 51 - protein, 24 aa, Artificial Sequence
  CD8a TM
IYIWAPLAGTCGVLLLSLVITLYC

SEQ ID NO: 52 - protein, 21 aa, Artificial Sequence
  CD8a TM
IYIWAPLAGTCGVLLLSLVIT

SEQ ID NO: 53 - protein, 112 aa, Homo sapiens
  CD3 zeta
RVKFSRSADAPAYQQGQNQLYNELNLGRREEYDVLDKRRGRDPEMGGKPRRKNPQEGLYNELQKDKMAEAYSEIGMKGERRRGKGHDGLYQGLSTATKDTYDALHMQALPPR

SEQ ID NO: 54 - protein, 112 aa, Homo sapiens
  CD3 zeta
RVKFSRSAEPPAYQQGQNQLYNELNLGRREEYDVLDKRRGRDPEMGGKPRRKNPQEGLYNELQKDKMAEAYSEIGMKGERRRGKGHDGLYQGLSTATKDTYDALHMQALPPR

SEQ ID NO: 55 - protein, 112 aa, Homo sapiens
  CD3 zeta
RVKFSRSADAPAYKQGQNQLYNELNLGRREEYDVLDKRRGRDPEMGGKPRRKNPQEGLYNELQKDKMAEAYSEIGMKGERRRGKGHDGLYQGLSTATKDTYDALHMQALPPR

SEQ ID NO: 56 - protein, 42 aa, Homo sapiens
  4-1BB (amino acids 214-255)
KRGRKKLLYIFKQPFMRPVQTTQEEDGCSCRFPEEEEGGCEL

SEQ ID NO: 57 - protein, 27 aa, Homo sapiens
  CD28 (amino acids 153-179)
FWVLVVVGGVLACYSLLVTVAFIIFWV

SEQ ID NO: 58 - protein, 66 aa, Homo sapiens
  CD28 (amino acids 114-179)
IEVMYPPPYLDNEKSNGTIIHVKGKHLCPSPLFPGPSKPFWVLVVVGGVLACYSLLVTVAFIIFWV

SEQ ID NO: 59 - protein, 41 aa, Homo sapiens
  CD28 (amino acids 180-220)
RSKRSRLLHSDYMNMTPRRPGPTRKHYQPYAPPRDFAAYRS

SEQ ID NO: 60 - protein, 41 aa, Homo sapiens
  CD28 (LL to GG)
RSKRSRGGHSDYMNMTPRRPGPTRKHYQPYAPPRDFAAYRS

SEQ ID NO: 61 - protein, 18 aa, Artificial Sequence
  T2A
EGRGSLLTCGDVEENPGP

SEQ ID NO: 62 - protein, 24 aa, Artificial Sequence
  T2A
LEGGGEGRGSLLTCGDVEENPGPR

SEQ ID NO: 63 - protein, 22 aa, Artificial Sequence
  P2A
GSGATNFSLLKQAGDVEENPGP

SEQ ID NO: 64 - protein, 19 aa, Artificial Sequence
  P2A
ATNFSLLKQAGDVEENPGP

SEQ ID NO: 65 - protein, 20 aa, Artificial Sequence
  E2A
QCTNYALLKLAGDVESNPGP

SEQ ID NO: 66 - protein, 22 aa, Artificial Sequence
  F2A
VKQTLNFDLLKLAGDVESNPGP

SEQ ID NO: 67 - protein, 128 aa, Artificial Sequence
  CAR-B  Light chain
MALPVTALLLPLALLLHAARPDIQMTQTTSSLSASLGDRVTISCRASQDISKYLNWYQQKPDGTVKLLIYHTSRLHSGVPSRFSGSGSGTDYSLTISNLEQEDIATYFCQQGNTLPYTFGGGTKLEIT

SEQ ID NO: 68 - protein, 165 aa, Artificial Sequence
  CAR-B Heavy chain
EVKLQESGPGLVAPSQSLSVTCTVSGVSLPDYGVSWIRQPPRKGLEWLGVIWGSETTYYNSALKSRLTIIKDNSKSQVFLKMNSLQTDDTAIYYCAKHYYYGGSYAMDYWGQGTSVTVSSTTTPAPRPPTPAPTIASQPLSLRPEACRPAAGGAVHTRGLDFACD

SEQ ID NO: 69 - protein, 5 aa, Artificial Sequence
  CAR-B Heavy chain CDR1
DYGVS

SEQ ID NO: 70 - protein, 16 aa, Artificial Sequence
  CAR-B Heavy chain CDR2
VIWGSETTYYNSALKS

SEQ ID NO: 71 - protein, 12 aa, Artificial Sequence
  CAR-B Heavy chain CDR3
HYYYGGSYAMDY

SEQ ID NO: 72 - protein, 11 aa, Artificial Sequence
  CAR-B Light chain CDR1
RASQDISKYLN

SEQ ID NO: 73 - protein, 7 aa, Artificial Sequence
  CAR-B Light chain CDR2
HTSRLHS

SEQ ID NO: 74 - protein, 9 aa, Artificial Sequence
  CAR-B Light chain CDR3
QQGNTLPYT

SEQ ID NO: 75 - protein, 128 aa, Artificial Sequence
  CAR-A  Light chain
MALPVTALLLPLALLLHAARPDIAMTQSQKFMSTSVGDRVSVTCKASQNVDTNVAWYQQKPGQSPKALIYSASYRYSGVPDRFTGSGSGTDFTLTINNVQSEDLAEYFCQQYNNYPFTFGSGTKLEIK

SEQ ID NO: 76 - protein, 167 aa, Artificial Sequence
  CAR-A Heavy chain
DVQLVESGGGLVQPGGSRKLSCAASGFTFSSFGMHWVRQAPEKGLEWVAYISSDSSAIYYADTVKGRFTISRDNPKNTLFLQMTSLRSEDTAMYYCGRGRENIYYGSRLDYWGQGTTLTVSSTTTPAPRPPTPAPTIASQPLSLRPEACRPAAGGAVHTRGLDFACD

SEQ ID NO: 77 - protein, 5 aa, Artificial Sequence
  CAR-A Heavy chain CDR1
SFGMH

SEQ ID NO: 78 - protein, 17 aa, Artificial Sequence
  CAR-A Heavy chain CDR2
YISSDSSAIYYADTVKG

SEQ ID NO: 79 - protein, 13 aa, Artificial Sequence
  CAR-A Heavy chain CDR3
GRENIYYGSRLDY

SEQ ID NO: 80 - protein, 11 aa, Artificial Sequence
  CAR-A Light chain CDR1
KASQNVDTNVA

SEQ ID NO: 81 - protein, 7 aa, Artificial Sequence
  CAR-A Light chain CDR2
SASYRYS

SEQ ID NO: 82 - protein, 9 aa, Artificial Sequence
  CAR-A Light chain CDR3
QQYNNYPFT

SEQ ID NO: 83 - protein, 308 aa, Artificial Sequence
  CAR-B scFv
MALPVTALLLPLALLLHAARPDIQMTQTTSSLSASLGDRVTISCRASQDISKYLNWYQQKPDGTVKLLIYHTSRLHSGVPSRFSGSGSGTDYSLTISNLEQEDIATYFCQQGNTLPYTFGGGTKLEITGGGGSGGGGSGGGGSEVKLQESGPGLVAPSQSLSVTCTVSGVSLPDYGVSWIRQPPRKGLEWLGVIWGSETTYYNSALKSRLTIIKDNSKSQVFLKMNSLQTDDTAIYYCAKHYYYGGSYAMDYWGQGTSVTVSSTTTPAPRPPTPAPTIASQPLSLRPEACRPAAGGAVHTRGLDFACD

SEQ ID NO: 84 - protein, 315 aa, Artificial Sequence
  CAR-A scFv
MALPVTALLLPLALLLHAARPDIAMTQSQKFMSTSVGDRVSVTCKASQNVDTNVAWYQQKPGQSPKALIYSASYRYSGVPDRFTGSGSGTDFTLTINNVQSEDLAEYFCQQYNNYPFTFGSGTKLEIKGGGGSGGGGSGGGGSGGGGSDVQLVESGGGLVQPGGSRKLSCAASGFTFSSFGMHWVRQAPEKGLEWVAYISSDSSAIYYADTVKGRFTISRDNPKNTLFLQMTSLRSEDTAMYYCGRGRENIYYGSRLDYWGQGTTLTVSSTTTPAPRPPTPAPTIASQPLSLRPEACRPAAGGAVHTRGLDFACD

SEQ ID NO: 85 - protein, 10 aa, Artificial Sequence
  linker
GGGGSGGGGS

SEQ ID NO: 86 - protein, 4 aa, Artificial Sequence
  TGFBR2 cyto domain 4 aa
CYRV

SEQ ID NO: 87 - protein, 13 aa, Artificial Sequence
  Partial of TGFBR2 extracellular domain
TIPPHVQKSVNND

SEQ ID NO: 88 - protein, 5 aa, Artificial Sequence
  Linker
AAGSG

SEQ ID NO: 89 - protein, 3 aa, Artificial Sequence
  Linker
GSG

SEQ ID NO: 90 - protein, 320 aa, Artificial Sequence
  CTSR-1A
LQCFCHLCTKDNFTCVTDGLCFVSVTETTDKVIHNSMCIAEIDLIPRDRPFVCAPSSKTGSVTTTYCCNQDHCNKIELPTTVKSSPGLGPVELAAVIAGPVCFVCISLMLMVYICHNRTVIHHRVPNEEDPSLDRPFISEGTTLKDLIYDAAGGPGAGSAAPVSSTSSLPLAALNMRVRRRLSLFLNVRTQVAADWTALAEEMDFEYLEIRQLETQADPTGRLLDAWQGRPGASVGRLLELLTKLGRDDVLLELGPSIEEDCQKYILKQQQEEAEKPLQVAAVDSSVPRTAELAGITTLDDPLGHMPERFDAFICYCPSD

SEQ ID NO: 91 - protein, 294 aa, Artificial Sequence
  CTSR-1B
LQCFCHLCTKDNFTCVTDGLCFVSVTETTDKVIHNSMCIAEIDLIPRDRPFVCAPSSKTGSVTTTYCCNQDHCNKIELPTTVKSSPGLGPVELAAVIAGPVCFVCISLMLMVYIGGGGSGGGGSAAGGPGAGSAAPVSSTSSLPLAALNMRVRRRLSLFLNVRTQVAADWTALAEEMDFEYLEIRQLETQADPTGRLLDAWQGRPGASVGRLLELLTKLGRDDVLLELGPSIEEDCQKYILKQQQEEAEKPLQVAAVDSSVPRTAELAGITTLDDPLGHMPERFDAFICYCPSD

SEQ ID NO: 92 - protein, 346 aa, Artificial Sequence
  CTSR-2A
TIPPHVQKSVNNDMIVTDNNGAVKFPQLCKFCDVRFSTCDNQKSCMSNCSITSICEKPQEVCVAVWRKNDENITLETVCHDPKLPYHDFILEDAASPKCIMKEKKKPGETFFMCSCSSDECNDNIIFSEEYNTSNPDLLLVIFQVTGISLLPPLGVAISVIIIFYCYRVNRQQKLSAAGGPGAGSAAPVSSTSSLPLAALNMRVRRRLSLFLNVRTQVAADWTALAEEMDFEYLEIRQLETQADPTGRLLDAWQGRPGASVGRLLELLTKLGRDDVLLELGPSIEEDCQKYILKQQQEEAEKPLQVAAVDSSVPRTAELAGITTLDDPLGHMPERFDAFICYCPSD

SEQ ID NO: 93 - protein, 516 aa, Artificial Sequence
  CTSR-2B
TIPPHVQKSVNNDMIVTDNNGAVKFPQLCKFCDVRFSTCDNQKSCMSNCSITSICEKPQEVCVAVWRKNDENITLETVCHDPKLPYHDFILEDAASPKCIMKEKKKPGETFFMCSCSSDECNDNIIFSEEYNTSNPDLLLVIFQVTGISLLPPLGVAISVIIIFYCYRVNRQQKLSAAGGPGAGSAAPVSSTSSLPLAALNMRVRRRLSLFLNVRTQVAADWTALAEEMDFEYLEIRQLETQADPTGRLLDAWQGRPGASVGRLLELLTKLGRDDVLLELGPSIEEDCQKYILKQQQEEAEKPLQVAAVDSSVPRTAELAGITTLDDPLGHMPERFDAFICYCPSDAAGGPGAGSAAPVSSTSSLPLAALNMRVRRRLSLFLNVRTQVAADWTALAEEMDFEYLEIRQLETQADPTGRLLDAWQGRPGASVGRLLELLTKLGRDDVLLELGPSIEEDCQKYILKQQQEEAEKPLQVAAVDSSVPRTAELAGITTLDDPLGHMPERFDAFICYCPSD

SEQ ID NO: 94 - protein, 521 aa, Artificial Sequence
  CTSR-2C
TIPPHVQKSVNNDMIVTDNNGAVKFPQLCKFCDVRFSTCDNQKSCMSNCSITSICEKPQEVCVAVWRKNDENITLETVCHDPKLPYHDFILEDAASPKCIMKEKKKPGETFFMCSCSSDECNDNIIFSEEYNTSNPDLLLVIFQVTGISLLPPLGVAISVIIIFYCYRVNRQQKLSAAGGPGAGSAAPVSSTSSLPLAALNMRVRRRLSLFLNVRTQVAADWTALAEEMDFEYLEIRQLETQADPTGRLLDAWQGRPGASVGRLLELLTKLGRDDVLLELGPSIEEDCQKYILKQQQEEAEKPLQVAAVDSSVPRTAELAGITTLDDPLGHMPERFDAFICYCPSDGGGGSAAGGPGAGSAAPVSSTSSLPLAALNMRVRRRLSLFLNVRTQVAADWTALAEEMDFEYLEIRQLETQADPTGRLLDAWQGRPGASVGRLLELLTKLGRDDVLLELGPSIEEDCQKYILKQQQEEAEKPLQVAAVDSSVPRTAELAGITTLDDPLGHMPERFDAFICYCPSD

SEQ ID NO: 95 - protein, 169 aa, Artificial Sequence
  CTSR-2IN
TIPPHVQKSVNNDMIVTDNNGAVKFPQLCKFCDVRFSTCDNQKSCMSNCSITSICEKPQEVCVAVWRKNDENITLETVCHDPKLPYHDFILEDAASPKCIMKEKKKPGETFFMCSCSSDECNDNIIFSEEYNTSNPDLLLVIFQVTGISLLPPLGVAISVIIIFYCYRV

SEQ ID NO: 96 - protein, 199 aa, Artificial Sequence
  CTSR-2IN-T2A
TIPPHVQKSVNNDMIVTDNNGAVKFPQLCKFCDVRFSTCDNQKSCMSNCSITSICEKPQEVCVAVWRKNDENITLETVCHDPKLPYHDFILEDAASPKCIMKEKKKPGETFFMCSCSSDECNDNIIFSEEYNTSNPDLLLVIFQVTGISLLPPLGVAISVIIIFYCYRVNRQQKLSAAGSGEGRGSLLTCGDVEENPGP

SEQ ID NO: 97 - protein, 377 aa, Artificial Sequence
  CTSR-2EN
VTGISLLPPLGVAISVIIIFYCYRVNRQQKLSAAGGPGAGSAAPVSSTSSLPLAALNMRVRRRLSLFLNVRTQVAADWTALAEEMDFEYLEIRQLETQADPTGRLLDAWQGRPGASVGRLLELLTKLGRDDVLLELGPSIEEDCQKYILKQQQEEAEKPLQVAAVDSSVPRTAELAGITTLDDPLGHMPERFDAFICYCPSDGGGGSAAGGPGAGSAAPVSSTSSLPLAALNMRVRRRLSLFLNVRTQVAADWTALAEEMDFEYLEIRQLETQADPTGRLLDAWQGRPGASVGRLLELLTKLGRDDVLLELGPSIEEDCQKYILKQQQEEAEKPLQVAAVDSSVPRTAELAGITTLDDPLGHMPERFDAFICYCPSD

SEQ ID NO: 98 - protein, 542 aa, Artificial Sequence
  CTSR-2EN-T2A
TIPPHVQKSVNNDMIVTDNNGAVKFPQLCKFCDVRFSTCDNQKSCMSNCSITSICEKPQEVCVAVWRKNDENITLETVCHDPKLPYHDFILEDAASPKCIMKEKKKPGETFFMCSCSSDECNDNIIFSEEYNTSNPDLLLVIFQVTGISLLPPLGVAISVIIIFYCYRVNRQQKLSAAGGPGAGSAAPVSSTSSLPLAALNMRVRRRLSLFLNVRTQVAADWTALAEEMDFEYLEIRQLETQADPTGRLLDAWQGRPGASVGRLLELLTKLGRDDVLLELGPSIEEDCQKYILKQQQEEAEKPLQVAAVDSSVPRTAELAGITTLDDPLGHMPERFDAFICYCPSDGGGGSAAGGPGAGSAAPVSSTSSLPLAALNMRVRRRLSLFLNVRTQVAADWTALAEEMDFEYLEIRQLETQADPTGRLLDAWQGRPGASVGRLLELLTKLGRDDVLLELGPSIEEDCQKYILKQQQEEAEKPLQVAAVDSSVPRTAELAGITTLDDPLGHMPERFDAFICYCPSDGSGEGRGSLLTCGDVEENPGP

SEQ ID NO: 99 - protein, 367 aa, Artificial Sequence
  CTSR-2A-T2A
TIPPHVQKSVNNDMIVTDNNGAVKFPQLCKFCDVRFSTCDNQKSCMSNCSITSICEKPQEVCVAVWRKNDENITLETVCHDPKLPYHDFILEDAASPKCIMKEKKKPGETFFMCSCSSDECNDNIIFSEEYNTSNPDLLLVIFQVTGISLLPPLGVAISVIIIFYCYRVNRQQKLSAAGGPGAGSAAPVSSTSSLPLAALNMRVRRRLSLFLNVRTQVAADWTALAEEMDFEYLEIRQLETQADPTGRLLDAWQGRPGASVGRLLELLTKLGRDDVLLELGPSIEEDCQKYILKQQQEEAEKPLQVAAVDSSVPRTAELAGITTLDDPLGHMPERFDAFICYCPSDGSGEGRGSLLTCGDVEENPGP

SEQ ID NO: 100 - protein, 411 aa, Artificial Sequence
  CTSR-2EN-T2A
TIPPHVQKSVNNDVTGISLLPPLGVAISVIIIFYCYRVNRQQKLSAAGGPGAGSAAPVSSTSSLPLAALNMRVRRRLSLFLNVRTQVAADWTALAEEMDFEYLEIRQLETQADPTGRLLDAWQGRPGASVGRLLELLTKLGRDDVLLELGPSIEEDCQKYILKQQQEEAEKPLQVAAVDSSVPRTAELAGITTLDDPLGHMPERFDAFICYCPSDGGGGSAAGGPGAGSAAPVSSTSSLPLAALNMRVRRRLSLFLNVRTQVAADWTALAEEMDFEYLEIRQLETQADPTGRLLDAWQGRPGASVGRLLELLTKLGRDDVLLELGPSIEEDCQKYILKQQQEEAEKPLQVAAVDSSVPRTAELAGITTLDDPLGHMPERFDAFICYCPSDGSGEGRGSLLTCGDVEENPGP

SEQ ID NO: 101 - protein, 10 aa, Artificial Sequence
  Myc tag
EQKLISEEDL

SEQ ID NO: 102 - protein, 21 aa, Artificial Sequence
  CD8a signal peptide
MALPVTALLLPLALLLHAARP

SEQ ID NO: 103 - protein, 6 aa, Artificial Sequence
  His tag
HHHHHH

SEQ ID NO: 104 - protein, 1066 aa, Artificial Sequence
  CTSR-2C-T2A-CAR-A
MALPVTALLLPLALLLHAARPEQKLISEEDLTIPPHVQKSVNNDMIVTDNNGAVKFPQLCKFCDVRFSTCDNQKSCMSNCSITSICEKPQEVCVAVWRKNDENITLETVCHDPKLPYHDFILEDAASPKCIMKEKKKPGETFFMCSCSSDECNDNIIFSEEYNTSNPDLLLVIFQVTGISLLPPLGVAISVIIIFYCYRVNRQQKLSAAGGPGAGSAAPVSSTSSLPLAALNMRVRRRLSLFLNVRTQVAADWTALAEEMDFEYLEIRQLETQADPTGRLLDAWQGRPGASVGRLLELLTKLGRDDVLLELGPSIEEDCQKYILKQQQEEAEKPLQVAAVDSSVPRTAELAGITTLDDPLGHMPERFDAFICYCPSDGGGGSAAGGPGAGSAAPVSSTSSLPLAALNMRVRRRLSLFLNVRTQVAADWTALAEEMDFEYLEIRQLETQADPTGRLLDAWQGRPGASVGRLLELLTKLGRDDVLLELGPSIEEDCQKYILKQQQEEAEKPLQVAAVDSSVPRTAELAGITTLDDPLGHMPERFDAFICYCPSDGSGEGRGSLLTCGDVEENPGPMALPVTALLLPLALLLHAARPDIAMTQSQKFMSTSVGDRVSVTCKASQNVDTNVAWYQQKPGQSPKALIYSASYRYSGVPDRFTGSGSGTDFTLTINNVQSEDLAEYFCQQYNNYPFTFGSGTKLEIKGGGGSGGGGSGGGGSGGGGSDVQLVESGGGLVQPGGSRKLSCAASGFTFSSFGMHWVRQAPEKGLEWVAYISSDSSAIYYADTVKGRFTISRDNPKNTLFLQMTSLRSEDTAMYYCGRGRENIYYGSRLDYWGQGTTLTVSSTTTPAPRPPTPAPTIASQPLSLRPEACRPAAGGAVHTRGLDFACDIYIWAPLAGTCGVLLLSLVITLYCKRGRKKLLYIFKQPFMRPVQTTQEEDGCSCRFPEEEEGGCELRVKFSRSADAPAYKQGQNQLYNELNLGRREEYDVLDKRRGRDPEMGGKPRRKNPQEGLYNELQKDKMAEAYSEIGMKGERRRGKGHDGLYQGLSTATKDTYDALHMQALPPR

SEQ ID NO: 105 - protein, 1059 aa, Artificial Sequence
  CTSR-2C-T2A-CAR-B
MALPVTALLLPLALLLHAARPEQKLISEEDLTIPPHVQKSVNNDMIVTDNNGAVKFPQLCKFCDVRFSTCDNQKSCMSNCSITSICEKPQEVCVAVWRKNDENITLETVCHDPKLPYHDFILEDAASPKCIMKEKKKPGETFFMCSCSSDECNDNIIFSEEYNTSNPDLLLVIFQVTGISLLPPLGVAISVIIIFYCYRVNRQQKLSAAGGPGAGSAAPVSSTSSLPLAALNMRVRRRLSLFLNVRTQVAADWTALAEEMDFEYLEIRQLETQADPTGRLLDAWQGRPGASVGRLLELLTKLGRDDVLLELGPSIEEDCQKYILKQQQEEAEKPLQVAAVDSSVPRTAELAGITTLDDPLGHMPERFDAFICYCPSDGGGGSAAGGPGAGSAAPVSSTSSLPLAALNMRVRRRLSLFLNVRTQVAADWTALAEEMDFEYLEIRQLETQADPTGRLLDAWQGRPGASVGRLLELLTKLGRDDVLLELGPSIEEDCQKYILKQQQEEAEKPLQVAAVDSSVPRTAELAGITTLDDPLGHMPERFDAFICYCPSDGSGEGRGSLLTCGDVEENPGPMALPVTALLLPLALLLHAARPDIQMTQTTSSLSASLGDRVTISCRASQDISKYLNWYQQKPDGTVKLLIYHTSRLHSGVPSRFSGSGSGTDYSLTISNLEQEDIATYFCQQGNTLPYTFGGGTKLEITGGGGSGGGGSGGGGSEVKLQESGPGLVAPSQSLSVTCTVSGVSLPDYGVSWIRQPPRKGLEWLGVIWGSETTYYNSALKSRLTIIKDNSKSQVFLKMNSLQTDDTAIYYCAKHYYYGGSYAMDYWGQGTSVTVSSTTTPAPRPPTPAPTIASQPLSLRPEACRPAAGGAVHTRGLDFACDIYIWAPLAGTCGVLLLSLVITLYCKRGRKKLLYIFKQPFMRPVQTTQEEDGCSCRFPEEEEGGCELRVKFSRSADAPAYKQGQNQLYNELNLGRREEYDVLDKRRGRDPEMGGKPRRKNPQEGLYNELQKDKMAEAYSEIGMKGERRRGKGHDGLYQGLSTATKDTYDALHMQALPPR

SEQ ID NO: 106 - protein, 891 aa, Artificial Sequence
  CTSR-2A-T2A-CAR-A
MALPVTALLLPLALLLHAARPEQKLISEEDLTIPPHVQKSVNNDMIVTDNNGAVKFPQLCKFCDVRFSTCDNQKSCMSNCSITSICEKPQEVCVAVWRKNDENITLETVCHDPKLPYHDFILEDAASPKCIMKEKKKPGETFFMCSCSSDECNDNIIFSEEYNTSNPDLLLVIFQVTGISLLPPLGVAISVIIIFYCYRVNRQQKLSAAGGPGAGSAAPVSSTSSLPLAALNMRVRRRLSLFLNVRTQVAADWTALAEEMDFEYLEIRQLETQADPTGRLLDAWQGRPGASVGRLLELLTKLGRDDVLLELGPSIEEDCQKYILKQQQEEAEKPLQVAAVDSSVPRTAELAGITTLDDPLGHMPERFDAFICYCPSDGSGEGRGSLLTCGDVEENPGPMALPVTALLLPLALLLHAARPDIAMTQSQKFMSTSVGDRVSVTCKASQNVDTNVAWYQQKPGQSPKALIYSASYRYSGVPDRFTGSGSGTDFTLTINNVQSEDLAEYFCQQYNNYPFTFGSGTKLEIKGGGGSGGGGSGGGGSGGGGSDVQLVESGGGLVQPGGSRKLSCAASGFTFSSFGMHWVRQAPEKGLEWVAYISSDSSAIYYADTVKGRFTISRDNPKNTLFLQMTSLRSEDTAMYYCGRGRENIYYGSRLDYWGQGTTLTVSSTTTPAPRPPTPAPTIASQPLSLRPEACRPAAGGAVHTRGLDFACDIYIWAPLAGTCGVLLLSLVITLYCKRGRKKLLYIFKQPFMRPVQTTQEEDGCSCRFPEEEEGGCELRVKFSRSADAPAYKQGQNQLYNELNLGRREEYDVLDKRRGRDPEMGGKPRRKNPQEGLYNELQKDKMAEAYSEIGMKGERRRGKGHDGLYQGLSTATKDTYDALHMQALPPR

SEQ ID NO: 107 - protein, 884 aa, Artificial Sequence
  CTSR-2C-T2A-CAR-B
MALPVTALLLPLALLLHAARPEQKLISEEDLTIPPHVQKSVNNDMIVTDNNGAVKFPQLCKFCDVRFSTCDNQKSCMSNCSITSICEKPQEVCVAVWRKNDENITLETVCHDPKLPYHDFILEDAASPKCIMKEKKKPGETFFMCSCSSDECNDNIIFSEEYNTSNPDLLLVIFQVTGISLLPPLGVAISVIIIFYCYRVNRQQKLSAAGGPGAGSAAPVSSTSSLPLAALNMRVRRRLSLFLNVRTQVAADWTALAEEMDFEYLEIRQLETQADPTGRLLDAWQGRPGASVGRLLELLTKLGRDDVLLELGPSIEEDCQKYILKQQQEEAEKPLQVAAVDSSVPRTAELAGITTLDDPLGHMPERFDAFICYCPSDGSGEGRGSLLTCGDVEENPGPMALPVTALLLPLALLLHAARPDIQMTQTTSSLSASLGDRVTISCRASQDISKYLNWYQQKPDGTVKLLIYHTSRLHSGVPSRFSGSGSGTDYSLTISNLEQEDIATYFCQQGNTLPYTFGGGTKLEITGGGGSGGGGSGGGGSEVKLQESGPGLVAPSQSLSVTCTVSGVSLPDYGVSWIRQPPRKGLEWLGVIWGSETTYYNSALKSRLTIIKDNSKSQVFLKMNSLQTDDTAIYYCAKHYYYGGSYAMDYWGQGTSVTVSSTTTPAPRPPTPAPTIASQPLSLRPEACRPAAGGAVHTRGLDFACDIYIWAPLAGTCGVLLLSLVITLYCKRGRKKLLYIFKQPFMRPVQTTQEEDGCSCRFPEEEEGGCELRVKFSRSADAPAYKQGQNQLYNELNLGRREEYDVLDKRRGRDPEMGGKPRRKNPQEGLYNELQKDKMAEAYSEIGMKGERRRGKGHDGLYQGLSTATKDTYDALHMQALPPR

SEQ ID NO: 108 - protein, 723 aa, Artificial Sequence
  CTSR-2IN-T2A-CAR-A
MALPVTALLLPLALLLHAARPEQKLISEEDLTIPPHVQKSVNNDMIVTDNNGAVKFPQLCKFCDVRFSTCDNQKSCMSNCSITSICEKPQEVCVAVWRKNDENITLETVCHDPKLPYHDFILEDAASPKCIMKEKKKPGETFFMCSCSSDECNDNIIFSEEYNTSNPDLLLVIFQVTGISLLPPLGVAISVIIIFYCYRVNRQQKLSAAGSGEGRGSLLTCGDVEENPGPMALPVTALLLPLALLLHAARPDIAMTQSQKFMSTSVGDRVSVTCKASQNVDTNVAWYQQKPGQSPKALIYSASYRYSGVPDRFTGSGSGTDFTLTINNVQSEDLAEYFCQQYNNYPFTFGSGTKLEIKGGGGSGGGGSGGGGSGGGGSDVQLVESGGGLVQPGGSRKLSCAASGFTFSSFGMHWVRQAPEKGLEWVAYISSDSSAIYYADTVKGRFTISRDNPKNTLFLQMTSLRSEDTAMYYCGRGRENIYYGSRLDYWGQGTTLTVSSTTTPAPRPPTPAPTIASQPLSLRPEACRPAAGGAVHTRGLDFACDIYIWAPLAGTCGVLLLSLVITLYCKRGRKKLLYIFKQPFMRPVQTTQEEDGCSCRFPEEEEGGCELRVKFSRSADAPAYKQGQNQLYNELNLGRREEYDVLDKRRGRDPEMGGKPRRKNPQEGLYNELQKDKMAEAYSEIGMKGERRRGKGHDGLYQGLSTATKDTYDALHMQALPPR

SEQ ID NO: 109 - protein, 716 aa, Artificial Sequence
  CTSR-2IN-T2A-CAR-B
MALPVTALLLPLALLLHAARPEQKLISEEDLTIPPHVQKSVNNDMIVTDNNGAVKFPQLCKFCDVRFSTCDNQKSCMSNCSITSICEKPQEVCVAVWRKNDENITLETVCHDPKLPYHDFILEDAASPKCIMKEKKKPGETFFMCSCSSDECNDNIIFSEEYNTSNPDLLLVIFQVTGISLLPPLGVAISVIIIFYCYRVNRQQKLSAAGSGEGRGSLLTCGDVEENPGPMALPVTALLLPLALLLHAARPDIQMTQTTSSLSASLGDRVTISCRASQDISKYLNWYQQKPDGTVKLLIYHTSRLHSGVPSRFSGSGSGTDYSLTISNLEQEDIATYFCQQGNTLPYTFGGGTKLEITGGGGSGGGGSGGGGSEVKLQESGPGLVAPSQSLSVTCTVSGVSLPDYGVSWIRQPPRKGLEWLGVIWGSETTYYNSALKSRLTIIKDNSKSQVFLKMNSLQTDDTAIYYCAKHYYYGGSYAMDYWGQGTSVTVSSTTTPAPRPPTPAPTIASQPLSLRPEACRPAAGGAVHTRGLDFACDIYIWAPLAGTCGVLLLSLVITLYCKRGRKKLLYIFKQPFMRPVQTTQEEDGCSCRFPEEEEGGCELRVKFSRSADAPAYKQGQNQLYNELNLGRREEYDVLDKRRGRDPEMGGKPRRKNPQEGLYNELQKDKMAEAYSEIGMKGERRRGKGHDGLYQGLSTATKDTYDALHMQALPPR

SEQ ID NO: 110 - protein, 935 aa, Artificial Sequence
  CTSR-2EN-T2A-CAR-A
MALPVTALLLPLALLLHAARPEQKLISEEDLTIPPHVQKSVNNDVTGISLLPPLGVAISVIIIFYCYRVNRQQKLSAAGGPGAGSAAPVSSTSSLPLAALNMRVRRRLSLFLNVRTQVAADWTALAEEMDFEYLEIRQLETQADPTGRLLDAWQGRPGASVGRLLELLTKLGRDDVLLELGPSIEEDCQKYILKQQQEEAEKPLQVAAVDSSVPRTAELAGITTLDDPLGHMPERFDAFICYCPSDGGGGSAAGGPGAGSAAPVSSTSSLPLAALNMRVRRRLSLFLNVRTQVAADWTALAEEMDFEYLEIRQLETQADPTGRLLDAWQGRPGASVGRLLELLTKLGRDDVLLELGPSIEEDCQKYILKQQQEEAEKPLQVAAVDSSVPRTAELAGITTLDDPLGHMPERFDAFICYCPSDGSGEGRGSLLTCGDVEENPGPMALPVTALLLPLALLLHAARPDIAMTQSQKFMSTSVGDRVSVTCKASQNVDTNVAWYQQKPGQSPKALIYSASYRYSGVPDRFTGSGSGTDFTLTINNVQSEDLAEYFCQQYNNYPFTFGSGTKLEIKGGGGSGGGGSGGGGSGGGGSDVQLVESGGGLVQPGGSRKLSCAASGFTFSSFGMHWVRQAPEKGLEWVAYISSDSSAIYYADTVKGRFTISRDNPKNTLFLQMTSLRSEDTAMYYCGRGRENIYYGSRLDYWGQGTTLTVSSTTTPAPRPPTPAPTIASQPLSLRPEACRPAAGGAVHTRGLDFACDIYIWAPLAGTCGVLLLSLVITLYCKRGRKKLLYIFKQPFMRPVQTTQEEDGCSCRFPEEEEGGCELRVKFSRSADAPAYKQGQNQLYNELNLGRREEYDVLDKRRGRDPEMGGKPRRKNPQEGLYNELQKDKMAEAYSEIGMKGERRRGKGHDGLYQGLSTATKDTYDALHMQALPPR

SEQ ID NO: 111 - protein, 928 aa, Artificial Sequence
  CTSR-2EN-T2A-CAR-B
MALPVTALLLPLALLLHAARPEQKLISEEDLTIPPHVQKSVNNDVTGISLLPPLGVAISVIIIFYCYRVNRQQKLSAAGGPGAGSAAPVSSTSSLPLAALNMRVRRRLSLFLNVRTQVAADWTALAEEMDFEYLEIRQLETQADPTGRLLDAWQGRPGASVGRLLELLTKLGRDDVLLELGPSIEEDCQKYILKQQQEEAEKPLQVAAVDSSVPRTAELAGITTLDDPLGHMPERFDAFICYCPSDGGGGSAAGGPGAGSAAPVSSTSSLPLAALNMRVRRRLSLFLNVRTQVAADWTALAEEMDFEYLEIRQLETQADPTGRLLDAWQGRPGASVGRLLELLTKLGRDDVLLELGPSIEEDCQKYILKQQQEEAEKPLQVAAVDSSVPRTAELAGITTLDDPLGHMPERFDAFICYCPSDGSGEGRGSLLTCGDVEENPGPMALPVTALLLPLALLLHAARPDIQMTQTTSSLSASLGDRVTISCRASQDISKYLNWYQQKPDGTVKLLIYHTSRLHSGVPSRFSGSGSGTDYSLTISNLEQEDIATYFCQQGNTLPYTFGGGTKLEITGGGGSGGGGSGGGGSEVKLQESGPGLVAPSQSLSVTCTVSGVSLPDYGVSWIRQPPRKGLEWLGVIWGSETTYYNSALKSRLTIIKDNSKSQVFLKMNSLQTDDTAIYYCAKHYYYGGSYAMDYWGQGTSVTVSSTTTPAPRPPTPAPTIASQPLSLRPEACRPAAGGAVHTRGLDFACDIYIWAPLAGTCGVLLLSLVITLYCKRGRKKLLYIFKQPFMRPVQTTQEEDGCSCRFPEEEEGGCELRVKFSRSADAPAYKQGQNQLYNELNLGRREEYDVLDKRRGRDPEMGGKPRRKNPQEGLYNELQKDKMAEAYSEIGMKGERRRGKGHDGLYQGLSTATKDTYDALHMQALPPR

SEQ ID NO: 112 - DNA, 544 bp, Artificial Sequence
  Ef1alpha promoter with HTLV1 enhancer
ggatctgcgatcgctccggtgcccgtcagtgggcagagcgcacatcgcccacagtccccgagaagttggggggaggggtcggcaattgaaccggtgcctagagaaggtggcgcggggtaaactgggaaagtgatgtcgtgtactggctccgcctttttcccgagggtgggggagaaccgtatataagtgcagtagtcgccgtgaacgttctttttcgcaacgggtttgccgccagaacacagctgaagcttcgaggggctcgcatctctccttcacgcgcccgccgccctacctgaggccgccatccacgccggttgagtcgcgttctgccgcctcccgcctgtggtgcctcctgaactgcgtccgccgtctaggtaagtttaaagctcaggtcgagaccgggcctttgtccggcgctcccttggagcctacctagactcagccggctctccacgctttgcctgaccctgcttgctcaactctacgtctttgtttcgttttctgttctgcgccgttacagatccaagctgtgaccggcgcctac

SEQ ID NO: 113 - protein, 21 aa, Artificial Sequence
  T2A
GSGEGRGSLLTCGDVEENPGP

SEQ ID NO: 114 - protein, 23 aa, Artificial Sequence
  T2A
AAGSGEGRGSLLTCGDVEENPGP

SEQ ID NO: 115 - protein, 18 aa, Artificial Sequence
  Linker
GSTSGSGKPGSGEGSTKG

SEQ ID NO: 116 - protein, 21 aa, Artificial Sequence
  Linker
SRGGGGSGGGGSGGGGSLEMA

SEQ ID NO: 117 - protein, 465 aa, Artificial Sequence
  CAR-B (no signal peptide)
DIQMTQTTSSLSASLGDRVTISCRASQDISKYLNWYQQKPDGTVKLLIYHTSRLHSGVPSRFSGSGSGTDYSLTISNLEQEDIATYFCQQGNTLPYTFGGGTKLEITGGGGSGGGGSGGGGSEVKLQESGPGLVAPSQSLSVTCTVSGVSLPDYGVSWIRQPPRKGLEWLGVIWGSETTYYNSALKSRLTIIKDNSKSQVFLKMNSLQTDDTAIYYCAKHYYYGGSYAMDYWGQGTSVTVSSTTTPAPRPPTPAPTIASQPLSLRPEACRPAAGGAVHTRGLDFACDIYIWAPLAGTCGVLLLSLVITLYCKRGRKKLLYIFKQPFMRPVQTTQEEDGCSCRFPEEEEGGCELRVKFSRSADAPAYKQGQNQLYNELNLGRREEYDVLDKRRGRDPEMGGKPRRKNPQEGLYNELQKDKMAEAYSEIGMKGERRRGKGHDGLYQGLSTATKDTYDALHMQALPPR

SEQ ID NO: 118 - protein, 472 aa, Artificial Sequence
  CAR-A (no signal peptide)
DIAMTQSQKFMSTSVGDRVSVTCKASQNVDTNVAWYQQKPGQSPKALIYSASYRYSGVPDRFTGSGSGTDFTLTINNVQSEDLAEYFCQQYNNYPFTFGSGTKLEIKGGGGSGGGGSGGGGSGGGGSDVQLVESGGGLVQPGGSRKLSCAASGFTFSSFGMHWVRQAPEKGLEWVAYISSDSSAIYYADTVKGRFTISRDNPKNTLFLQMTSLRSEDTAMYYCGRGRENIYYGSRLDYWGQGTTLTVSSTTTPAPRPPTPAPTIASQPLSLRPEACRPAAGGAVHTRGLDFACDIYIWAPLAGTCGVLLLSLVITLYCKRGRKKLLYIFKQPFMRPVQTTQEEDGCSCRFPEEEEGGCELRVKFSRSADAPAYKQGQNQLYNELNLGRREEYDVLDKRRGRDPEMGGKPRRKNPQEGLYNELQKDKMAEAYSEIGMKGERRRGKGHDGLYQGLSTATKDTYDALHMQALPPR

SEQ ID NO: 119 - protein, 214 aa, Artificial Sequence
  IL10Ra Extracellular domain
HGTELPSPPSVWFEAEFFHHILHWTPIPNQSESTCYEVALLRYGIESWNSISNCSQTLSYDLTAVTLDLYHSNGYRARVRAVDGSRHSNWTVTNTRFSVDEVTLTVGSVNLEIHNGFILGKIQLPRPKMAPANDTYESIFSHFREYEIAIRKVPGNFTFTHKKVKHENFSLLTSGEVGEFCVQVKPSVASRSNKGMWSKEECISLTRQYFTVTN

SEQ ID NO: 120 - protein, 21 aa, Artificial Sequence
  IL10Ra Transmembrane domain
VIIFFAFVLLLSGALAYCLAL

SEQ ID NO: 121 - protein, 322 aa, Artificial Sequence
  IL10Ra Cytoplasmic  domain
QLYVRRRKKLPSVLLFKKPSPFIFISQRPSPETQDTIHPLDEEAFLKVSPELKNLDLHGSTDSGFGSTKPSLQTEEPQFLLPDPHPQADRTLGNREPPVLGDSCSSGSSNSTDSGICLQEPSLSPSTGPTWEQQVGSNSRGQDDSGIDLVQNSEGRAGDTQGGSALGHHSPPEPEVPGEEDPAAVAFQGYLRQTRCAEEKATKTGCLEEESPLTDGLGPKFGRCLVDEAGLHPPALAKGYLKQDPLEMTLASSGAPTGQWNQPTEEWSLLALSSCSDLGISDWSFAHDLAPLGCVAAPGGLLGSFNSDLVTLPLISSLQSSE

SEQ ID NO: 122 - protein, 201 aa, Artificial Sequence
  IL10Rb Extracellular domain
MVPPPENVRMNSVNFKNILQWESPAFAKGNLTFTAQYLSYRIFQDKCMNTTLTECDFSSLSKYGDHTLRVRAEFADEHSDWVNITFCPVDDTIIGPPGMQVEVLADSLHMRFLAPKIENEYETWTMKNVYNSWTYNVQYWKNGTDEKFQITPQYDFEVLRNLEPWTTYCVQVRGFLPDRNKAGEWSEPVCEQTTHDETVPS

SEQ ID NO: 123 - protein, 22 aa, Artificial Sequence
  IL10Rb Transmembrane domain
WMVAVILMASVFMVCLALLGCF

SEQ ID NO: 124 - protein, 83 aa, Artificial Sequence
  IL10Rb Cytoplasmic domain
ALLWCVYKKTKYAFSPRNSLPQHLKEFLGHPHHNTLLFFSFPLSDENDVFDKLSVIAEDSESGKQNPGDSCSLGTPPGQGPQS

SEQ ID NO: 125 - protein, 207 aa, Artificial Sequence
  IL4R Extracellular domain
MKVLQEPTCVSDYMSISTCEWKMNGPTNCSTELRLLYQLVFLLSEAHTCIPENNGGAGCVCHLLMDDVVSADNYTLDLWAGQQLLWKGSFKPSEHVKPRAPGNLTVHTNVSDTLLLTWSNPYPPDNYLYNHLTYAVNIWSENDPADFRIYNVTYLEPSLRIAASTLKSGISYRARVRAWAQCYNTTWSEWSPSTKWHNSYREPFEQH

SEQ ID NO: 126 - protein, 24 aa, Artificial Sequence
  IL4R Transmembrane domain
LLLGVSVSCIVILAVCLLCYVSIT

SEQ ID NO: 127 - protein, 569 aa, Artificial Sequence
  IL4R Cytoplasmic domain
KIKKEWWDQIPNPARSRLVAIIIQDAQGSQWEKRSRGQEPAKCPHWKNCLTKLLPCFLEHNMKRDEDPHKAAKEMPFQGSGKSAWCPVEISKTVLWPESISVVRCVELFEAPVECEEEEEVEEEKGSFCASPESSRDDFQEGREGIVARLTESLFLDLLGEENGGFCQQDMGESCLLPPSGSTSAHMPWDEFPSAGPKEAPPWGKEQPLHLEPSPPASPTQSPDNLTCTETPLVIAGNPAYRSFSNSLSQSPCPRELGPDPLLARHLEEVEPEMPCVPQLSEPTTVPQPEPETWEQILRRNVLQHGAAAAPVSAPTSGYQEFVHAVEQGGTQASAVVGLGPPGEAGYKAFSSLLASSAVSPEKCGFGASSGEEGYKPFQDLIPGCPGDPAPVPVPLFTFGLDREPPRSPQSSHLPSSSPEHLGLEPGEKVEDMPKPPLPQEQATDPLVDSLGSGIVYSALTCHLCGHLKQCHGQEDGGQTPVMASPCCGCCCGDRSSPPTTPLRAPDPSPGGVPLEASLCPASLAPSGISEKSKSSSSFHPAPGNAQSSSQTPKIVNFVSVGPTYMRVS

SEQ ID NO: 128 - protein, 296 aa, Artificial Sequence
  MyD88
MAAGGPGAGSAAPVSSTSSLPLAALNMRVRRRLSLFLNVRTQVAADWTALAEEMDFEYLEIRQLETQADPTGRLLDAWQGRPGASVGRLLELLTKLGRDDVLLELGPSIEEDCQKYILKQQQEEAEKPLQVAAVDSSVPRTAELAGITTLDDPLGHMPERFDAFICYCPSDIQFVQEMIRQLEQTNYRLKLCVSDRDVLPGTCVWSIASELIEKRCRRMVVVVSDDYLQSKECDFQTKFALSLSPGAHQKRLIPIKYKAMKKEFPSILRFITVCDYTNPCTKSWFWTRLAKALSLP

SEQ ID NO: 129 - protein, 380 aa, Artificial Sequence
  TGFBR2 Cytoplasmic domain
CYRVNRQQKLSSTWETGKTRKLMEFSEHCAIILEDDRSDISSTCANNINHNTELLPIELDTLVGKGRFAEVYKAKLKQNTSEQFETVAVKIFPYEEYASWKTEKDIFSDINLKHENILQFLTAEERKTELGKQYWLITAFHAKGNLQEYLTRHVISWEDLRKLGSSLARGIAHLHSDHTPCGRPKMPIVHRDLKSSNILVKNDLTCCLCDFGLSLRLDPTLSVDDLANSGQVGTARYMAPEVLESRMNLENVESFKQTDVYSMALVLWEMTSRCNAVGEVKDYEPPFGSKVREHPCVESMKDNVLRDRGRPEIPSFWLNHQGIQMVCETLTECWDHDPEARLTAQCVAERFSELEHLDRLSGRSCSEEKIPEDGSLNTTK

SEQ ID NO: 130 - protein, 356 aa, Artificial Sequence
  TGFBR1 Cytoplasmic domain
CHNRTVIHHRVPNEEDPSLDRPFISEGTTLKDLIYDMTTSGSGSGLPLLVQRTIARTIVLQESIGKGRFGEVWRGKWRGEEVAVKIFSSREERSWFREAEIYQTVMLRHENILGFIAADNKDNGTWTQLWLVSDYHEHGSLFDYLNRYTVTVEGMIKLALSTASGLAHLHMEIVGTQGKPAIAHRDLKSKNILVKKNGTCCIADLGLAVRHDSATDTIDIAPNHRVGTKRYMAPEVLDDSINMKHFESFKRADIYAMGLVFWEIARRCSIGGIHEDYQLPYYDLVPSDPSVEEMRKVVCEQKLRPNIPNRWQSCEALRVMAKIMRECWYANGAARLTALRIKKTLSQLSQQEGIKM